European Patent Specification EP 3 527 670 B1, published October 18, 2023. Title: MIRNA BIOGENESIS IN EXOSOMES FOR DIAGNOSIS AND THERAPY. Applicant: Board of Regents, The University of Texas System Beth Israel Deaconess Medical Center, Inc. KALLURI, Raghu MELO, Sonia. The sequence listing filed with the application follows.

SEQUENCE LISTING (56 sequences)

SEQ ID NO: 1 - DNA, 20 bp, Artificial sequence
  Synthetic primer
caggaggtggtgaaggacat

SEQ ID NO: 2 - DNA, 19 bp, Artificial sequence
  Synthetic primer
cccgttggtctgtgagttt

SEQ ID NO: 3 - DNA, 20 bp, Artificial sequence
  Synthetic primer
gataccctcccaatcccagt

SEQ ID NO: 4 - DNA, 20 bp, Artificial sequence
  Synthetic primer
gtcactgaccgcagagatga

SEQ ID NO: 5 - DNA, 21 bp, Artificial sequence
  Synthetic primer
agtggctgtcgggtattcatc

SEQ ID NO: 6 - DNA, 23 bp, Artificial sequence
  Synthetic primer
ccgtccatatcccttgaagaatc

SEQ ID NO: 7 - DNA, 19 bp, Artificial sequence
  Synthetic primer
gctggtggtaagcccagac

SEQ ID NO: 8 - DNA, 21 bp, Artificial sequence
  Synthetic primer
ggctcgctagtagagaccaaa

SEQ ID NO: 9 - DNA, 21 bp, Artificial sequence
  Synthetic primer
catgtacgttgctatccaggc

SEQ ID NO: 10 - DNA, 21 bp, Artificial sequence
  Synthetic primer
ctccttaatgtcacgcacgat

SEQ ID NO: 11 - DNA, 20 bp, Artificial sequence
  Synthetic primer
ggctgtattcccctccatcg

SEQ ID NO: 12 - DNA, 22 bp, Artificial sequence
  Synthetic primer
ccagttggtaacaatgccatgt

SEQ ID NO: 13 - DNA, 25 bp, Artificial sequence
  Synthetic primer
aggtagtaggttgtatagttttagg

SEQ ID NO: 14 - DNA, 25 bp, Artificial sequence
  Synthetic primer
taggaaagacagtagattgtatagt

SEQ ID NO: 15 - DNA, 21 bp, Artificial sequence
  Synthetic primer
agcacatcatggtttacatgc

SEQ ID NO: 16 - DNA, 23 bp, Artificial sequence
  Synthetic primer
ctagagcagcaaataatgattgg

SEQ ID NO: 17 - DNA, 24 bp, Artificial sequence
  Synthetic primer
ttcaagtaatccaggataggctgt

SEQ ID NO: 18 - DNA, 22 bp, Artificial sequence
  Synthetic primer
tgcaagtaaccaagaataggcc

SEQ ID NO: 19 - DNA, 20 bp, Artificial sequence
  Synthetic primer
tgagtgtgttttccctccct

SEQ ID NO: 20 - DNA, 17 bp, Artificial sequence
  Synthetic primer
gccatggctgctgtcag

SEQ ID NO: 21 - DNA, 20 bp, Artificial sequence
  Synthetic primer
gtccctgagaccctttaacc

SEQ ID NO: 22 - DNA, 19 bp, Artificial sequence
  Synthetic primer
aacctcacctgtgaccctg

SEQ ID NO: 23 - DNA, 20 bp, Artificial sequence
  Synthetic primer
gtccctgagaccctaacttg

SEQ ID NO: 24 - DNA, 18 bp, Artificial sequence
  Synthetic primer
agcctaacccgtggattt

SEQ ID NO: 25 - DNA, 17 bp, Artificial sequence
  Synthetic primer
ttccacagcagcccctg

SEQ ID NO: 26 - DNA, 18 bp, Artificial sequence
  Synthetic primer
gatgtgcctcggtggtgt

SEQ ID NO: 27 - DNA, 20 bp, Artificial sequence
  Synthetic primer
ctcgtcttacccagcagtgt

SEQ ID NO: 28 - DNA, 24 bp, Artificial sequence
  Synthetic primer
gtcatcattaccaggcagtattag

SEQ ID NO: 29 - DNA, 23 bp, Artificial sequence
  Synthetic primer
gtcaagagcaataacgaaaaatg

SEQ ID NO: 30 - DNA, 21 bp, Artificial sequence
  Synthetic primer
gaggtcaggagcaataatgaa

SEQ ID NO: 31 - DNA, 23 bp, Artificial sequence
  Synthetic primer
taccctgtagatccgaatttgtg

SEQ ID NO: 32 - DNA, 24 bp, Artificial sequence
  Synthetic primer
attcccctagatacgaatttgtga

SEQ ID NO: 33 - DNA, 23 bp, Artificial sequence
  Synthetic primer
gcttatcagactgatgttgactg

SEQ ID NO: 34 - DNA, 17 bp, Artificial sequence
  Synthetic primer
cagcccatcgactggtg

SEQ ID NO: 35 - DNA, 18 bp, Artificial sequence
  Synthetic primer
gcagggcttagctgcttg

SEQ ID NO: 36 - DNA, 19 bp, Artificial sequence
  Synthetic primer
ggcggaacttagccactgt

SEQ ID NO: 37 - DNA, 22 bp, Artificial sequence
  Synthetic primer
gttaatgctaatcgtgataggg

SEQ ID NO: 38 - DNA, 24 bp, Artificial sequence
  Synthetic primer
gctaatatgtaggagtcagttgga

SEQ ID NO: 39 - DNA, 18 bp, Artificial sequence
  Synthetic primer
ctcaaaatgggggcgctt

SEQ ID NO: 40 - DNA, 20 bp, Artificial sequence
  Synthetic primer
caccccaaaatcgaagcact

SEQ ID NO: 41 - DNA, 21 bp, Artificial sequence
  Synthetic primer
ccaccccgttctacatacttc

SEQ ID NO: 42 - DNA, 20 bp, Artificial sequence
  Synthetic primer
accgtaccgagctgcatact

SEQ ID NO: 43 - DNA, 21 bp, Artificial Sequence
  Synthetic probe
cacaaattcggttctacaggg

SEQ ID NO: 44 - DNA, 22 bp, Artificial sequence
  Synthetic probe
tcaacatcagtctgataagcta

SEQ ID NO: 45 - DNA, 20 bp, Artificial sequence
  Synthetic probe
agtatgcagctcggtacggt

SEQ ID NO: 46 - DNA, 40 bp, Artificial sequence
  Synthetic probe
tgaagtttttgcatcgaccatatattcccctagaatcgaa

SEQ ID NO: 47 - DNA, 36 bp, Artificial sequence
  Synthetic probe
tgtcagacagcccatcgactggtgttgccatgagat

SEQ ID NO: 48 - DNA, 25 bp, Artificial sequence
  Synthetic probe
cagcacgcttccgctgcgccactct

SEQ ID NO: 49 - DNA, 21 bp, Artificial sequence
  Synthetic oligo
ggaacgagcccaaguacaatt

SEQ ID NO: 50 - DNA, 21 bp, Artificial sequence
  Synthetic oligo
uuguacuugggcucguuccgg

SEQ ID NO: 51 - DNA, 21 bp, Artificial sequence
  Synthetic oligo
guuuaucauucaaguguaatt

SEQ ID NO: 52 - DNA, 21 bp, Artificial sequence
  Synthetic oligo
uuacacuugaaugauaaactg

SEQ ID NO: 53 - DNA, 21 bp, Artificial sequence
  Synthetic oligo
ggagagccuuuggucucuatt

SEQ ID NO: 54 - DNA, 21 bp, Artificial sequence
  Synthetic oligo
uagagaccaaaggcucuccgg

SEQ ID NO: 55 - DNA, 21 bp, Artificial sequence
  Synthetic oligo
ggcguuacacgaugcacuutt

SEQ ID NO: 56 - DNA, 21 bp, Artificial sequence
  Synthetic oligo
aagugcaucguguaacgcctg